European Patent Application EP 4 265 717 A1, published October 25, 2023. Title: 一种鼠抗MCR-1/MCR-2蛋白杂交瘤细胞株，单克隆抗体及应用. Applicant: 天津一瑞生物科技股份有限公司. The sequence listing filed with the application follows.

SEQUENCE LISTING (20 sequences)

SEQ ID NO: 1 - protein, 11 aa, Artificial sequence
RASQDINNYLN

SEQ ID NO: 2 - protein, 7 aa, Artificial sequence
YTSRLHS

SEQ ID NO: 3 - protein, 10 aa, Artificial sequence
QQGKTIHPWT

SEQ ID NO: 4 - protein, 11 aa, Artificial sequence
GYSITSDYAWN

SEQ ID NO: 5 - protein, 16 aa, Artificial sequence
QISDSAVTTYNPSLKS

SEQ ID NO: 6 - protein, 11 aa, Artificial sequence
RNFYGYNFFDY

SEQ ID NO: 7 - protein, 110 aa, Artificial sequence
DIQMTQTTSSLSASLGDRVTINCRASQDINNYLNWYQQKPDGTVKLLIYYTSRLHSGVPSRFSGSGSRTDYSLTISNLEREDIATYFCQQGKTIHPWTFGGGTKLDIKRA

SEQ ID NO: 8 - DNA, 330 bp, Artificial sequence
  source 1..330: mol_type = other DNA
gatatccagatgacacagactacatcctccctgtctgcctctctgggagacagagtcaccatcaattgcagggcaagtcaggacattaacaattatttaaactggtatcagcagaaaccagatggaactgttaaactcctgatctactacacttcaagattacattcaggagtcccatcaaggttcagcggcagtgggtctagaacagattattctctcaccattagcaacctggaacgagaagatattgccacttacttttgccaacagggtaaaacgattcatccgtggacgttcggtggaggcaccaagctggacatcaaacgggct

SEQ ID NO: 9 - protein, 121 aa, Artificial sequence
VKLQESGPGLVKPSQSLSLTCTVTGYSITSDYAWNWIRQFPGNKLEWMGQISDSAVTTYNPSLKSRISINRDTSKNQFFLQLNSVTPEDTATYYCARRNFYGYNFFDYWGRGTSLTVSSAK

SEQ ID NO: 10 - DNA, 363 bp, Artificial sequence
  source 1..363: mol_type = other DNA
gtgaagctgcaggagtcaggacctggcctggtgaaaccttctcagtctctgtccctcacctgcactgtcactggctactcaatcaccagtgattatgcctggaactggatccggcagtttccaggaaacaaactggagtggatgggccagataagcgacagtgctgtcactacctacaacccatctctcaaaagtcgaatctctatcaatcgagacacatccaagaaccagttcttcctgcagttgaattctgtgactcctgaggacacagccacatattactgtgcaagaaggaacttctacgggtacaatttttttgactactggggccgaggcacctctctcactgtctcttcagccaaa

SEQ ID NO: 11 - protein, 16 aa, Artificial sequence
RSSQNIVCSYGNPCLE

SEQ ID NO: 12 - protein, 7 aa, Artificial sequence
KVSNRFS

SEQ ID NO: 13 - protein, 9 aa, Artificial sequence
FQSSHVPWT

SEQ ID NO: 14 - protein, 10 aa, Artificial sequence
GYTFTSYVMH

SEQ ID NO: 15 - protein, 17 aa, Artificial sequence
YFNPYNDGANYNEKFKG

SEQ ID NO: 16 - protein, 10 aa, Artificial sequence
GPYGNYAMDY

SEQ ID NO: 17 - protein, 113 aa, Artificial sequence
DVLMTQTPLSLPVSLGDQASISCRSSQNIVCSYGNPCLEWYLQKPGQSPKLLIYKVSNRFSGVPDRFSGSGSGTDFTLKISRVEAEDLGVYYCFQSSHVPWTFGGGTELEIKR

SEQ ID NO: 18 - DNA, 339 bp, Artificial sequence
  source 1..339: mol_type = other DNA
gatgttttgatgacccagacgccactctccctgcctgtcagtcttggagatcaagcctccatctcttgcagatctagtcagaacattgtatgtagttatggaaacccctgtttagaatggtacctgcagaaaccaggccagtctccaaagctcctgatctacaaagtttccaaccgattttctggggtcccagacaggttcagtggcagtggatcagggacagatttcacactcaagatcagcagagtggaggctgaggatctgggagtttattactgctttcaaagttcacatgttccgtggacgttcggtggaggcaccgagctggaaatcaaacgg

SEQ ID NO: 19 - protein, 119 aa, Artificial sequence
VKLQQSGPELVKPGASVKMSCRASGYTFTSYVMHWVKQKPGQGLEWIGYFNPYNDGANYNEKFKGKATLSSDKSSGTAYMDLSSLTSEDSAVYYCARGPYGNYAMDYWGQGTSVTVSSA

SEQ ID NO: 20 - DNA, 357 bp, Artificial sequence
  source 1..357: mol_type = other DNA
gtgaagctgcagcagtctggacctgagctggtaaagcctggggcttcagtgaagatgtcctgcagggcttctggatacacattcactagctatgttatgcactgggtgaagcagaagcctgggcagggccttgagtggattggatattttaatccttacaatgacggtgctaactacaatgagaagttcaaaggcaaggccacactgtcttcagacaaatcctccggcacagcctatatggacctcagcagcctgacctctgaggactctgcggtctattattgtgcgagaggcccctatggtaactatgctatggactactggggtcaaggaacctcagtcaccgtctcctcagcc